European Patent Specification EP 3 969 575 B1, published January 1, 2025. Title: PHI29 DNA POLYMERASE MUTANTS WITH IMPROVED PRIMER RECOGNITION. Applicant: 4BASEBIO SL. Application US62/849,252. The sequence listing filed with the application follows.

SEQUENCE LISTING (6 sequences)

SEQ ID NO: 1 - protein, 575 aa, Bacillus subtilis [sequence omitted]

SEQ ID NO: 2 - protein, 575 aa, Artificial Sequence
  K64R Phi29DNApol mutant
MKHMPRKMYSCDFETTTKVEDCRVWAYGYMNIEDHSEYKIGNSLDEFMAWVLKVQADLYFHNLRFDGAFIINWLERNGFKWSADGLPNTYNTIISRMGQWYMIDICLGYKGKRKIHTVIYDSLKKLPFPVKKIAKDFKLTVLKGDIDYHKERPVGYKITPEEYAYIKNDIQIIAEALLIQFKQGLDRMTAGSDSLKGFKDIITTKKFKKVFPTLSLGLDKEVRYAYRGGFTWLNDRFKEKEIGEGMVFDVNSLYPAQMYSRLLPYGEPIVFEGKYVWDEDYPLHIQHIRCEFELKEGYIPTIQIKRSRFYKGNEYLKSSGGEIADLWLSNVDLELMKEHYDLYNVEYISGLKFKATTGLFKDFIDKWTYIKTTSEGAIKQLAKLMLNSLYGKFASNPDVTGKVPYLKENGALGFRLGEEETKDPVYTPMGVFITAWARYTTITAAQACYDRIIYCDTDSIHLTGTEIPDVIKDIVDPKKLGYWAHESTFKRAKYLRQKTYIQDIYMKEVDGKLVEGSPDDYTDIKFSVKCAGMTDKIKKEVTFENFKVGFSRKMKPKPVQVPGGVVLVDDTFTIK

SEQ ID NO: 3 - protein, 575 aa, Artificial Sequence
  M97K Phi29DNApol mutant
MKHMPRKMYSCDFETTTKVEDCRVWAYGYMNIEDHSEYKIGNSLDEFMAWVLKVQADLYFHNLKFDGAFIINWLERNGFKWSADGLPNTYNTIISRKGQWYMIDICLGYKGKRKIHTVIYDSLKKLPFPVKKIAKDFKLTVLKGDIDYHKERPVGYKITPEEYAYIKNDIQIIAEALLIQFKQGLDRMTAGSDSLKGFKDIITTKKFKKVFPTLSLGLDKEVRYAYRGGFTWLNDRFKEKEIGEGMVFDVNSLYPAQMYSRLLPYGEPIVFEGKYVWDEDYPLHIQHIRCEFELKEGYIPTIQIKRSRFYKGNEYLKSSGGEIADLWLSNVDLELMKEHYDLYNVEYISGLKFKATTGLFKDFIDKWTYIKTTSEGAIKQLAKLMLNSLYGKFASNPDVTGKVPYLKENGALGFRLGEEETKDPVYTPMGVFITAWARYTTITAAQACYDRIIYCDTDSIHLTGTEIPDVIKDIVDPKKLGYWAHESTFKRAKYLRQKTYIQDIYMKEVDGKLVEGSPDDYTDIKFSVKCAGMTDKIKKEVTFENFKVGFSRKMKPKPVQVPGGVVLVDDTFTIK

SEQ ID NO: 4 - protein, 575 aa, Artificial Sequence
  K64R / M97K Phi29DNApol double mutant
MKHMPRKMYSCDFETTTKVEDCRVWAYGYMNIEDHSEYKIGNSLDEFMAWVLKVQADLYFHNLRFDGAFIINWLERNGFKWSADGLPNTYNTIISRKGQWYMIDICLGYKGKRKIHTVIYDSLKKLPFPVKKIAKDFKLTVLKGDIDYHKERPVGYKITPEEYAYIKNDIQIIAEALLIQFKQGLDRMTAGSDSLKGFKDIITTKKFKKVFPTLSLGLDKEVRYAYRGGFTWLNDRFKEKEIGEGMVFDVNSLYPAQMYSRLLPYGEPIVFEGKYVWDEDYPLHIQHIRCEFELKEGYIPTIQIKRSRFYKGNEYLKSSGGEIADLWLSNVDLELMKEHYDLYNVEYISGLKFKATTGLFKDFIDKWTYIKTTSEGAIKQLAKLMLNSLYGKFASNPDVTGKVPYLKENGALGFRLGEEETKDPVYTPMGVFITAWARYTTITAAQACYDRIIYCDTDSIHLTGTEIPDVIKDIVDPKKLGYWAHESTFKRAKYLRQKTYIQDIYMKEVDGKLVEGSPDDYTDIKFSVKCAGMTDKIKKEVTFENFKVGFSRKMKPKPVQVPGGVVLVDDTFTIK

SEQ ID NO: 5 - DNA, 15 bp, Artificial Sequence
  5'-labelled primer of DNA duplex
gatcacagtgagtac

SEQ ID NO: 6 - DNA, 28 bp, Artificial Sequence
  template of DNA duplex
agaagtgtatctggtactcactgtgatc